European Patent Specification EP 4 341 390 B1, published July 1, 2026. Title: METHODS FOR MAKING LIBRARIES FOR NUCLEIC ACID SEQUENCING. Applicant: Becton, Dickinson and Company Godinez, Alvaro. The sequence listing filed with the application follows.

SEQUENCE LISTING (45 sequences)

SEQ ID NO: 1 - DNA, 12339 bp, Artificial Sequence
  3XFlag-Cas9-Fl26-Tn5
atacactccgctatcgctacgtgactgggtcatggctgcgccccgacacccgccaacacccgctgacgcgccctgacgggcttgtctgctcccggcatccgcttacagacaagctgtgaccgtctccgggagctgcatgtgtcagaggttttcaccgtcatcaccgaaacgcgcgaggcagctgcggtaaagctcatcagcgtggtcgtgcagcgattcacagatgtctgcctgttcatccgcgtccagctcgttgagtttctccagaagcgttaatgtctggcttctgataaagcgggccatgttaagggcggttttttcctgtttggtcactgatgcctccgtgtaagggggatttctgttcatgggggtaatgataccgatgaaacgagagaggatgctcacgatacgggttactgatgatgaacatgcccggttactggaacgttgtgagggtaaacaactggcggtatggatgcggcgggaccagagaaaaatcactcagggtcaatgccagccgaacgccagcaagacgtagcccagcgcgtcggccgccatgccggcgataatggcctgcttctcgccgaaacgtttggtggcgggaccagtgacgaaggcttgagcgagggcgtgcaagattccgaataccgcaagcgacaggccgatcatcgtcgcgctccagcgaaagcggtcctcgccgaaaatgacccagagcgctgccggcacctgtcctacgagttgcatgataaagaagacagtcataagtgcggcgacgatagtcatgccccgcgcccaccggaaggagctgactgggttgaaggctctcaagggcatcggtcgagatcccggtgcctaatgagtgagctaacttacattaattgcgttgcgctcactgcccgctttccagtcgggaaacctgtcgtgccagctgcattaatgaatcggccaacgcgcggggagaggcggtttgcgtattgggcgccagggtggtttttcttttcaccagtgagacgggcaacagctgattgcccttcaccgcctggccctgagagagttgcagcaagcggtccacgctggtttgccccagcaggcgaaaatcctgtttgatggtggttaacggcgggatataacatgagctgtcttcggtatcgtcgtatcccactaccgagatatccgcaccaacgcgcagcccggactcggtaatggcgcgcattgcgcccagcgccatctgatcgttggcaaccagcatcgcagtgggaacgatgccctcattcagcatttgcatggtttgttgaaaaccggacatggcactccagtcgccttcccgttccgctatcggctgaatttgattgcgagtgagatatttatgccagccagccagacgcagacgcgccgagacagaacttaatgggcccgctaacagcgcgatttgctggtgacccaatgcgaccagatgctccacgcccagtcgcgtaccgtcttcatgggagaaaataatactgttgatgggtgtctggtcagagacatcaagaaataacgccggaacattagtgcaggcagcttccacagcaatggcatcctggtcatccagcggatagttaatgatcagcccactgacgcgttgcgcgagaagattgtgcaccgccgctttacaggcttcgacgccgcttcgttctaccatcgacaccaccacgctggcacccagttgatcggcgcgagatttaatcgccgcgacaatttgcgacggcgcgtgcagggccagactggaggtggcaacgccaatcagcaacgactgtttgcccgccagttgttgtgccacgcggttgggaatgtaattcagctccgccatcgccgcttccactttttcccgcgttttcgcagaaacgtggctggcctggttcaccacgcgggaaacggtctgataagagacaccggcatactctgcgacatcgtataacgttactggtttcacattcaccaccctgaattgactctcttccgggcgctatcatgccataccgcgaaaggttttgcgccattcgatggtgtccgggatctcgacgctctcccttatgcgactcctgcattaggaagcagcccagtagtaggttgaggccgttgagcaccgccgccgcaaggaatggtgcatgccggcatgccgccctttcgtcttcaagaattaattcccaattccccaggcatcaaataaaacgaaaggctcagtcgaaagactgggcctttcgttttatctgttgtttgtcggtgaacgctctcctgagtaggacaaatccgccgggagcggatttgaacgttgcgaagcaacggcccggagggtggcgggcaggacgcccgccataaactgccaggaattaattccccaggcatcaaataaaacgaaaggctcagtcgaaagactgggcctttcgttttatctgttgtttgtcggtgaacgctctcctgagtaggacaaatccgccgggagcggatttgaacgttgcgaagcaacggcccggagggtggcgggcaggacgcccgccataaactgccaggaattaattccccaggcatcaaataaaacgaaaggctcagtcgaaagactgggcctttcgttttatctgttgtttgtcggtgaacgctctcctgagtaggacaaatccgccgggagcggatttgaacgttgcgaagcaacggcccggagggtggcgggcaggacgcccgccataaactgccaggaattaattccccaggcatcaaataaaacgaaaggctcagtcgaaagactgggcctttcgttttatctgttgtttgtcggtgaacgctctcctgagtaggacaaatccgccgggagcggatttgaacgttgcgaagcaacggcccggagggtggcgggcaggacgcccgccataaactgccaggaattaattccccaggcatcaaataaaacgaaaggctcagtcgaaagactgggcctttcgttttatctgttgtttgtcggtgaacgctctcctgagtaggacaaatccgccgggagcggatttgaacgttgcgaagcaacggcccggagggtggcgggcaggacgcccgccataaactgccaggaattggggatcggaattaattcccggtttaaaccggggatctcgatcccgcgaaattaatacgactcactataggggaattgtgagcggataacaattcccctctagaaataattttgtttaactttaagaaggagatataccatgggtgattacaaggatcacgatggcgattacaaggatcacgatatcgattacaaggatgatgatgataagatggataaaaagtattctattggtttagctatcggcacaaatagcgtcggatgggcggtgatcactgatgaatataaggttccgtctaaaaagttcaaggttctgggaaatacagaccgccacagtatcaaaaaaaatcttataggggctcttttatttgacagtggagagacagcggaagcgactcgtctcaaacggacagctcgtagaaggtatacacgtcggaagaatcgtatttgttatctacaggagattttttcaaatgagatggcgaaagtagatgatagtttctttcatcgacttgaagagtcttttttggtggaagaagacaagaagcatgaacgtcatcctatttttggaaatatagtagatgaagttgcttatcatgagaaatatccaactatctatcatctgcgaaaaaaattggtagattctactgataaagcggatttgcgcttaatctatttggccttagcgcatatgattaagtttcgtggtcattttttgattgagggagatttaaatcctgataatagtgatgtggacaaactatttatccagttggtacaaacctacaatcaattatttgaagaaaaccctattaacgcaagtggagtagatgctaaagcgattctttctgcacgattgagtaaatcaagacgattagaaaatctcattgctcagctccccggtgagaagaaaaatggcttatttgggaatctcattgctttgtcattgggtttgacccctaattttaaatcaaattttgatttggcagaagatgctaaattacagctttcaaaagatacttacgatgatgatttagataatttattggcgcaaattggagatcaatatgctgatttgtttttggcagctaagaatttatcagatgctattttactttcagatatcctaagagtaaatactgaaataactaaggctcccctatcagcatcaatgattaaacgctacgatgaacatcatcaagacttgactcttttaaaagctttagttcgacaacaacttccagaaaagtataaagaaatcttttttgatcaatcaaaaaacggatatgcaggttatattgatgggggagctagccaagaagaattttataaatttatcaaaccaattttagaaaaaatggatggtactgaggaattattggtgaaactaaatcgtgaagatttgctgcgcaagcaacggacctttgacaacggctctattccccatcaaattcacttgggtgagctgcatgctattttgagaagacaagaagacttttatccatttttaaaagacaatcgtgagaagattgaaaaaatcttgacttttcgaattccttattatgttggtccattggcgcgtggcaatagtcgttttgcatggatgactcggaagtctgaagaaacaattaccccatggaattttgaagaagttgtcgataaaggtgcttcagctcaatcatttattgaacgcatgacaaactttgataaaaatcttccaaatgaaaaagtactaccaaaacatagtttgctttatgagtattttacggtttataacgaattgacaaaggtcaaatatgttactgaaggaatgcgaaaaccagcatttctttcaggtgaacagaagaaagccattgttgatttactcttcaaaacaaatcgaaaagtaaccgttaagcaattaaaagaagattatttcaaaaaaatagaatgttttgatagtgttgaaatttcaggagttgaagatagatttaatgcttcattaggtacctaccatgatttgctaaaaattattaaagataaagattttttggataatgaagaaaatgaagatatcttagaggatattgttttaacattgaccttatttgaagatagggagatgattgaggaaagacttaaaacatatgctcacctctttgatgataaggtgatgaaacagcttaaacgtcgccgttatactggttggggacgtttgtctcgaaaattgattaatggtattagggataagcaatctggcaaaacaatattagattttttgaaatcagatggttttgccaatcgcaattttatgcagctgatccatgatgatagtttgacatttaaagaagacattcaaaaagcacaagtgtctggacaaggcgatagtttacatgaacatattgcaaatttagctggtagccctgctattaaaaaaggtattttacagactgtaaaagttgttgatgaattggtcaaagtaatggggcggcataagccagaaaatatcgttattgaaatggcacgtgaaaatcagacaactcaaaagggccagaaaaattcgcgagagcgtatgaaacgaatcgaagaaggtatcaaagaattaggaagtcagattcttaaagagcatcctgttgaaaatactcaattgcaaaatgaaaagctctatctctattatctccaaaatggaagagacatgtatgtggaccaagaattagatattaatcgtttaagtgattatgatgtcgatgccattgttccacaaagtttccttaaagacgattcaatagacaataaggtcttaacgcgttctgataaaaatcgtggtaaatcggataacgttccaagtgaagaagtagtcaaaaagatgaaaaactattggagacaacttctaaacgccaagttaatcactcaacgtaagtttgataatttaacgaaagctgaacgtggaggtttgagtgaacttgataaagctggttttatcaaacgccaattggttgaaactcgccaaatcactaagcatgtggcacaaattttggatagtcgcatgaatactaaatacgatgaaaatgataaacttattcgagaggttaaagtgattaccttaaaatctaaattagtttctgacttccgaaaagatttccaattctataaagtacgtgagattaacaattaccatcatgcccatgatgcgtatctaaatgccgtcgttggaactgctttgattaagaaatatccaaaacttgaatcggagtttgtctatggtgattataaagtttatgatgttcgtaaaatgattgctaagtctgagcaagaaataggcaaagcaaccgcaaaatatttcttttactctaatatcatgaacttcttcaaaacagaaattacacttgcaaatggagagattcgcaaacgccctctaatcgaaactaatggggaaactggagaaattgtctgggataaagggcgagattttgccacagtgcgcaaagtattgtccatgccccaagtcaatattgtcaagaaaacagaagtacagacaggcggattctccaaggagtcaattttaccaaaaagaaattcggacaagcttattgctcgtaaaaaagactgggatccaaaaaaatatggtggttttgatagtccaacggtagcttattcagtcctagtggttgctaaggtggaaaaagggaaatcgaagaagttaaaatccgttaaagagttactagggatcacaattatggaaagaagttcctttgaaaaaaatccgattgactttttagaagctaaaggatataaggaagttaaaaaagacttaatcattaaactacctaaatatagtctttttgagttagaaaacggtcgtaaacggatgctggctagtgccggagaattacaaaaaggaaatgagctggctctgccaagcaaatatgtgaattttttatatttagctagtcattatgaaaagttgaagggtagtccagaagataacgaacaaaaacaattgtttgtggagcagcataagcattatttagatgagattattgagcaaatcagtgaattttctaagcgtgttattttagcagatgccaatttagataaagttcttagtgcatataacaaacatagagacaaaccaatacgtgaacaagcagaaaatattattcatttatttacgttgacgaatcttggagctcccgctgcttttaaatattttgatacaacaattgatcgtaaacgatatacgtctacaaaagaagttttagatgccactcttatccatcaatccatcactggtctttatgaaacacgcattgatttgagtcagctaggaggtgacgatgacgataaagaattcggtggcggtggctctggcggtggtgggagtggaggtgggggatcaggaggaggcggttcccatatgattaccagtgcactgcatcgtgcggcggattgggcgaaaagcgtgttttctagtgctgcgctgggtgatccgcgtcgtaccgcgcgtctggtgaatgttgcggcgcaactggccaaatatagcggcaaaagcattaccattagcagcgaaggcagcaaagccatgcaggaaggcgcgtatcgttttattcgtaatccgaacgtgagcgcggaagcgattcgtaaagcgggtgccatgcagaccgtgaaactggcccaggaatttccggaactgctggcaattgaagataccacctctctgagctatcgtcatcaggtggcggaagaactgggcaaactgggtagcattcaggataaaagccgtggttggtgggtgcatagcgtgctgctgctggaagcgaccacctttcgtaccgtgggcctgctgcatcaagaatggtggatgcgtccggatgatccggcggatgcggatgaaaaagaaagcggcaaatggctggccgctgctgcaacttcgcgtctgagaatgggcagcatgatgagcaacgtgattgcggtgtgcgatcgtgaagcggatattcatgcgtatctgcaagataaactggcccataacgaacgttttgtggtgcgtagcaaacatccgcgtaaagatgtggaaagcggcctgtatctgtatgatcacctgaaaaaccagccggaactgggcggctatcagattagcattccgcagaaaggcgtggtggataaacgtggcaaacgtaaaaaccgtccggcgcgtaaagcgagcctgagcctgcgtagcggccgtattaccctgaaacagggcaacattaccctgaacgcggtgctggccgaagaaattaatccgccgaaaggcgaaaccccgctgaaatggctgctgctgaccagcgagccggtggaaagtctggcccaagcgctgcgtgtgattgatatttatacccatcgttggcgcattgaagaatttcacaaagcgtggaaaacgggtgcgggtgcggaacgtcagcgtatggaagaaccggataacctggaacgtatggtgagcattctgagctttgtggcggtgcgtctgctgcaactgcgtgaatcttttactccgccgcaagcactgcgtgcgcagggcctgctgaaagaagcggaacacgttgaaagccagagcgcggaaaccgtgctgaccccggatgaatgccaactgctgggctatctggataaaggcaaacgcaaacgcaaagaaaaagcgggcagcctgcaatgggcgtatatggcgattgcgcgtctgggcggctttatggatagcaaacgtaccggcattgcgagctggggtgcgctgtgggaaggttgggaagcgctgcaaagcaaactggatggctttctggccgcgaaagacctgatggcgcagggcattaaaatctgcatcacgggagatgcactagttgccctacccgagggcgagtcggtacgcatcgccgacatcgtgccgggtgcgcggcccaacagtgacaacgccatcgacctgaaagtccttgaccggcatggcaatcccgtgctcgccgaccggctgttccactccggcgagcatccggtgtacacggtgcgtacggtcgaaggtctgcgtgtgacgggcaccgcgaaccacccgttgttgtgtttggtcgacgtcgccggggtgccgaccctgctgtggaagctgatcgacgaaatcaagccgggcgattacgcggtgattcaacgcagcgcattcagcgtcgactgtgcaggttttgcccgcgggaaacccgaatttgcgcccacaacctacacagtcggcgtccctggactggtgcgtttcttggaagcacaccaccgagacccggacgcccaagctatcgccgacgagctgaccgacgggcggttctactacgcgaaagtcgccagtgtcaccgacgccggcgtgcagccggtgtatagccttcgtgtcgacacggcagaccacgcgtttatcacgaacgggttcgtcagccacgctactggcctcaccggtctgaactcaggcctcacgacaaatcctggtgtatccgcttggcaggtcaacacagcttatactgcgggacaattggtcacatataacggcaagacgtataaatgtttgcagccccacacctccttggcaggatgggaaccatccaacgttcctgccttgtggcagcttcaatgactgcaggaaggggatccggctgctaacaaagcccgaaaggaagctgagttggctgctgccaccgctgagcaataactagcataaccccttggggcctctaaacgggtcttgaggggttttttgctgaaaggaggaactatatccggataactacgtcaggtggcacttttcggggaaatgtgcgcggaacccctatttgtttatttttctaaatacattcaaatatgtatccgctcatgagacaataaccctgataaatgcttcaataatattgaaaaaggaagagtatgagtattcaacatttccgtgtcgcccttattcccttttttgcggcattttgccttcctgtttttgctcacccagaaacgctggtgaaagtaaaagatgctgaagatcagttgggtgcacgagtgggttacatcgaactggatctcaacagcggtaagatccttgagagttttcgccccgaagaacgtttcccaatgatgagcacttttaaagttctgctatgtggcgcggtattatcccgtgttgacgccgggcaagagcaactcggtcgccgcatacactattctcagaatgacttggttgagtactcaccagtcacagaaaagcatcttacggatggcatgacagtaagagaattatgcagtgctgccataaccatgagtgataacactgcggccaacttacttctgacaacgatcggaggaccgaaggagctaaccgcttttttgcacaacatgggggatcatgtaactcgccttgatcgttgggaaccggagctgaatgaagccataccaaacgacgagcgtgacaccacgatgcctgtagcaatggcaacaacgttgcgcaaactattaactggcgaactacttactctagcttcccggcaacaattaatagactggatggaggcggataaagttgcaggaccacttctgcgctcggcccttccggctggctggtttattgctgataaatctggagccggtgagcgtgggtctcgcggtatcattgcagcactggggccagatggtaagccctcccgtatcgtagttatctacacgacggggagtcaggcaactatggatgaacgaaatagacagatcgctgagataggtgcctcactgattaagcattggtaactgtcagaccaagtttactcatatatactttagattgatttaccccggttgataatcagaaaagccccaaaaacaggaagattgtataagcaaatatttaaattgtaaacgttaatattttgttaaaattcgcgttaaatttttgttaaatcagctcattttttaaccaataggccgaaatcggcaaaatcccttataaatcaaaagaatagcccgagatagggttgagtgttgttccagtttggaacaagagtccactattaaagaacgtggactccaacgtcaaagggcgaaaaaccgtctatcagggcgatggcccactacgtgaaccatcacccaaatcaagttttttggggtcgaggtgccgtaaagcactaaatcggaaccctaaagggagcccccgatttagagcttgacggggaaagccggcgaacgtggcgagaaaggaagggaagaaagcgaaaggagcgggcgctagggcgctggcaagtgtagcggtcacgctgcgcgtaaccaccacacccgccgcgcttaatgcgccgctacagggcgcgtaaaaggatctaggtgaagatcctttttgataatctcatgaccaaaatcccttaacgtgagttttcgttccactgagcgtcagaccccgtagaaaagatcaaaggatcttcttgagatcctttttttctgcgcgtaatctgctgcttgcaaacaaaaaaaccaccgctaccagcggtggtttgtttgccggatcaagagctaccaactctttttccgaaggtaactggcttcagcagagcgcagataccaaatactgtccttctagtgtagccgtagttaggccaccacttcaagaactctgtagcaccgcctacatacctcgctctgctaatcctgttaccagtggctgctgccagtggcgataagtcgtgtcttaccgggttggactcaagacgatagttaccggataaggcgcagcggtcgggctgaacggggggttcgtgcacacagcccagcttggagcgaacgacctacaccgaactgagatacctacagcgtgagctatgagaaagcgccacgcttcccgaagggagaaaggcggacaggtatccggtaagcggcagggtcggaacaggagagcgcacgagggagcttccagggggaaacgcctggtatctttatagtcctgtcgggtttcgccacctctgacttgagcgtcgatttttgtgatgctcgtcaggggggcggagcctatggaaaaacgccagcaacgcggcctttttacggttcctggccttttgctggccttttgctcacatgttctttcctgcgttatcccctgattctgtggataaccgtattaccgcctttgagtgagctgataccgctcgccgcagccgaacgaccgagcgcagcgagtcagtgagcgaggaagctatggtgcactctcagtacaatctgctctgatgccgcatagttaagccagt

SEQ ID NO: 2 - DNA, 12306 bp, Artificial Sequence
  3XFlag-Cas9-xTen-Tn5
atacactccgctatcgctacgtgactgggtcatggctgcgccccgacacccgccaacacccgctgacgcgccctgacgggcttgtctgctcccggcatccgcttacagacaagctgtgaccgtctccgggagctgcatgtgtcagaggttttcaccgtcatcaccgaaacgcgcgaggcagctgcggtaaagctcatcagcgtggtcgtgcagcgattcacagatgtctgcctgttcatccgcgtccagctcgttgagtttctccagaagcgttaatgtctggcttctgataaagcgggccatgttaagggcggttttttcctgtttggtcactgatgcctccgtgtaagggggatttctgttcatgggggtaatgataccgatgaaacgagagaggatgctcacgatacgggttactgatgatgaacatgcccggttactggaacgttgtgagggtaaacaactggcggtatggatgcggcgggaccagagaaaaatcactcagggtcaatgccagccgaacgccagcaagacgtagcccagcgcgtcggccgccatgccggcgataatggcctgcttctcgccgaaacgtttggtggcgggaccagtgacgaaggcttgagcgagggcgtgcaagattccgaataccgcaagcgacaggccgatcatcgtcgcgctccagcgaaagcggtcctcgccgaaaatgacccagagcgctgccggcacctgtcctacgagttgcatgataaagaagacagtcataagtgcggcgacgatagtcatgccccgcgcccaccggaaggagctgactgggttgaaggctctcaagggcatcggtcgagatcccggtgcctaatgagtgagctaacttacattaattgcgttgcgctcactgcccgctttccagtcgggaaacctgtcgtgccagctgcattaatgaatcggccaacgcgcggggagaggcggtttgcgtattgggcgccagggtggtttttcttttcaccagtgagacgggcaacagctgattgcccttcaccgcctggccctgagagagttgcagcaagcggtccacgctggtttgccccagcaggcgaaaatcctgtttgatggtggttaacggcgggatataacatgagctgtcttcggtatcgtcgtatcccactaccgagatatccgcaccaacgcgcagcccggactcggtaatggcgcgcattgcgcccagcgccatctgatcgttggcaaccagcatcgcagtgggaacgatgccctcattcagcatttgcatggtttgttgaaaaccggacatggcactccagtcgccttcccgttccgctatcggctgaatttgattgcgagtgagatatttatgccagccagccagacgcagacgcgccgagacagaacttaatgggcccgctaacagcgcgatttgctggtgacccaatgcgaccagatgctccacgcccagtcgcgtaccgtcttcatgggagaaaataatactgttgatgggtgtctggtcagagacatcaagaaataacgccggaacattagtgcaggcagcttccacagcaatggcatcctggtcatccagcggatagttaatgatcagcccactgacgcgttgcgcgagaagattgtgcaccgccgctttacaggcttcgacgccgcttcgttctaccatcgacaccaccacgctggcacccagttgatcggcgcgagatttaatcgccgcgacaatttgcgacggcgcgtgcagggccagactggaggtggcaacgccaatcagcaacgactgtttgcccgccagttgttgtgccacgcggttgggaatgtaattcagctccgccatcgccgcttccactttttcccgcgttttcgcagaaacgtggctggcctggttcaccacgcgggaaacggtctgataagagacaccggcatactctgcgacatcgtataacgttactggtttcacattcaccaccctgaattgactctcttccgggcgctatcatgccataccgcgaaaggttttgcgccattcgatggtgtccgggatctcgacgctctcccttatgcgactcctgcattaggaagcagcccagtagtaggttgaggccgttgagcaccgccgccgcaaggaatggtgcatgccggcatgccgccctttcgtcttcaagaattaattcccaattccccaggcatcaaataaaacgaaaggctcagtcgaaagactgggcctttcgttttatctgttgtttgtcggtgaacgctctcctgagtaggacaaatccgccgggagcggatttgaacgttgcgaagcaacggcccggagggtggcgggcaggacgcccgccataaactgccaggaattaattccccaggcatcaaataaaacgaaaggctcagtcgaaagactgggcctttcgttttatctgttgtttgtcggtgaacgctctcctgagtaggacaaatccgccgggagcggatttgaacgttgcgaagcaacggcccggagggtggcgggcaggacgcccgccataaactgccaggaattaattccccaggcatcaaataaaacgaaaggctcagtcgaaagactgggcctttcgttttatctgttgtttgtcggtgaacgctctcctgagtaggacaaatccgccgggagcggatttgaacgttgcgaagcaacggcccggagggtggcgggcaggacgcccgccataaactgccaggaattaattccccaggcatcaaataaaacgaaaggctcagtcgaaagactgggcctttcgttttatctgttgtttgtcggtgaacgctctcctgagtaggacaaatccgccgggagcggatttgaacgttgcgaagcaacggcccggagggtggcgggcaggacgcccgccataaactgccaggaattaattccccaggcatcaaataaaacgaaaggctcagtcgaaagactgggcctttcgttttatctgttgtttgtcggtgaacgctctcctgagtaggacaaatccgccgggagcggatttgaacgttgcgaagcaacggcccggagggtggcgggcaggacgcccgccataaactgccaggaattggggatcggaattaattcccggtttaaaccggggatctcgatcccgcgaaattaatacgactcactataggggaattgtgagcggataacaattcccctctagaaataattttgtttaactttaagaaggagatataccatgggtgattacaaggatcacgatggcgattacaaggatcacgatatcgattacaaggatgatgatgataagatggataaaaagtattctattggtttagctatcggcacaaatagcgtcggatgggcggtgatcactgatgaatataaggttccgtctaaaaagttcaaggttctgggaaatacagaccgccacagtatcaaaaaaaatcttataggggctcttttatttgacagtggagagacagcggaagcgactcgtctcaaacggacagctcgtagaaggtatacacgtcggaagaatcgtatttgttatctacaggagattttttcaaatgagatggcgaaagtagatgatagtttctttcatcgacttgaagagtcttttttggtggaagaagacaagaagcatgaacgtcatcctatttttggaaatatagtagatgaagttgcttatcatgagaaatatccaactatctatcatctgcgaaaaaaattggtagattctactgataaagcggatttgcgcttaatctatttggccttagcgcatatgattaagtttcgtggtcattttttgattgagggagatttaaatcctgataatagtgatgtggacaaactatttatccagttggtacaaacctacaatcaattatttgaagaaaaccctattaacgcaagtggagtagatgctaaagcgattctttctgcacgattgagtaaatcaagacgattagaaaatctcattgctcagctccccggtgagaagaaaaatggcttatttgggaatctcattgctttgtcattgggtttgacccctaattttaaatcaaattttgatttggcagaagatgctaaattacagctttcaaaagatacttacgatgatgatttagataatttattggcgcaaattggagatcaatatgctgatttgtttttggcagctaagaatttatcagatgctattttactttcagatatcctaagagtaaatactgaaataactaaggctcccctatcagcatcaatgattaaacgctacgatgaacatcatcaagacttgactcttttaaaagctttagttcgacaacaacttccagaaaagtataaagaaatcttttttgatcaatcaaaaaacggatatgcaggttatattgatgggggagctagccaagaagaattttataaatttatcaaaccaattttagaaaaaatggatggtactgaggaattattggtgaaactaaatcgtgaagatttgctgcgcaagcaacggacctttgacaacggctctattccccatcaaattcacttgggtgagctgcatgctattttgagaagacaagaagacttttatccatttttaaaagacaatcgtgagaagattgaaaaaatcttgacttttcgaattccttattatgttggtccattggcgcgtggcaatagtcgttttgcatggatgactcggaagtctgaagaaacaattaccccatggaattttgaagaagttgtcgataaaggtgcttcagctcaatcatttattgaacgcatgacaaactttgataaaaatcttccaaatgaaaaagtactaccaaaacatagtttgctttatgagtattttacggtttataacgaattgacaaaggtcaaatatgttactgaaggaatgcgaaaaccagcatttctttcaggtgaacagaagaaagccattgttgatttactcttcaaaacaaatcgaaaagtaaccgttaagcaattaaaagaagattatttcaaaaaaatagaatgttttgatagtgttgaaatttcaggagttgaagatagatttaatgcttcattaggtacctaccatgatttgctaaaaattattaaagataaagattttttggataatgaagaaaatgaagatatcttagaggatattgttttaacattgaccttatttgaagatagggagatgattgaggaaagacttaaaacatatgctcacctctttgatgataaggtgatgaaacagcttaaacgtcgccgttatactggttggggacgtttgtctcgaaaattgattaatggtattagggataagcaatctggcaaaacaatattagattttttgaaatcagatggttttgccaatcgcaattttatgcagctgatccatgatgatagtttgacatttaaagaagacattcaaaaagcacaagtgtctggacaaggcgatagtttacatgaacatattgcaaatttagctggtagccctgctattaaaaaaggtattttacagactgtaaaagttgttgatgaattggtcaaagtaatggggcggcataagccagaaaatatcgttattgaaatggcacgtgaaaatcagacaactcaaaagggccagaaaaattcgcgagagcgtatgaaacgaatcgaagaaggtatcaaagaattaggaagtcagattcttaaagagcatcctgttgaaaatactcaattgcaaaatgaaaagctctatctctattatctccaaaatggaagagacatgtatgtggaccaagaattagatattaatcgtttaagtgattatgatgtcgatgccattgttccacaaagtttccttaaagacgattcaatagacaataaggtcttaacgcgttctgataaaaatcgtggtaaatcggataacgttccaagtgaagaagtagtcaaaaagatgaaaaactattggagacaacttctaaacgccaagttaatcactcaacgtaagtttgataatttaacgaaagctgaacgtggaggtttgagtgaacttgataaagctggttttatcaaacgccaattggttgaaactcgccaaatcactaagcatgtggcacaaattttggatagtcgcatgaatactaaatacgatgaaaatgataaacttattcgagaggttaaagtgattaccttaaaatctaaattagtttctgacttccgaaaagatttccaattctataaagtacgtgagattaacaattaccatcatgcccatgatgcgtatctaaatgccgtcgttggaactgctttgattaagaaatatccaaaacttgaatcggagtttgtctatggtgattataaagtttatgatgttcgtaaaatgattgctaagtctgagcaagaaataggcaaagcaaccgcaaaatatttcttttactctaatatcatgaacttcttcaaaacagaaattacacttgcaaatggagagattcgcaaacgccctctaatcgaaactaatggggaaactggagaaattgtctgggataaagggcgagattttgccacagtgcgcaaagtattgtccatgccccaagtcaatattgtcaagaaaacagaagtacagacaggcggattctccaaggagtcaattttaccaaaaagaaattcggacaagcttattgctcgtaaaaaagactgggatccaaaaaaatatggtggttttgatagtccaacggtagcttattcagtcctagtggttgctaaggtggaaaaagggaaatcgaagaagttaaaatccgttaaagagttactagggatcacaattatggaaagaagttcctttgaaaaaaatccgattgactttttagaagctaaaggatataaggaagttaaaaaagacttaatcattaaactacctaaatatagtctttttgagttagaaaacggtcgtaaacggatgctggctagtgccggagaattacaaaaaggaaatgagctggctctgccaagcaaatatgtgaattttttatatttagctagtcattatgaaaagttgaagggtagtccagaagataacgaacaaaaacaattgtttgtggagcagcataagcattatttagatgagattattgagcaaatcagtgaattttctaagcgtgttattttagcagatgccaatttagataaagttcttagtgcatataacaaacatagagacaaaccaatacgtgaacaagcagaaaatattattcatttatttacgttgacgaatcttggagctcccgctgcttttaaatattttgatacaacaattgatcgtaaacgatatacgtctacaaaagaagttttagatgccactcttatccatcaatccatcactggtctttatgaaacacgcattgatttgagtcagctaggaggtgacagcggttccgaaactcccggtacatcagaaagcgcgacccccgaaagcatgattaccagtgcactgcatcgtgcggcggattgggcgaaaagcgtgttttctagtgctgcgctgggtgatccgcgtcgtaccgcgcgtctggtgaatgttgcggcgcaactggccaaatatagcggcaaaagcattaccattagcagcgaaggcagcaaagccatgcaggaaggcgcgtatcgttttattcgtaatccgaacgtgagcgcggaagcgattcgtaaagcgggtgccatgcagaccgtgaaactggcccaggaatttccggaactgctggcaattgaagataccacctctctgagctatcgtcatcaggtggcggaagaactgggcaaactgggtagcattcaggataaaagccgtggttggtgggtgcatagcgtgctgctgctggaagcgaccacctttcgtaccgtgggcctgctgcatcaagaatggtggatgcgtccggatgatccggcggatgcggatgaaaaagaaagcggcaaatggctggccgctgctgcaacttcgcgtctgagaatgggcagcatgatgagcaacgtgattgcggtgtgcgatcgtgaagcggatattcatgcgtatctgcaagataaactggcccataacgaacgttttgtggtgcgtagcaaacatccgcgtaaagatgtggaaagcggcctgtatctgtatgatcacctgaaaaaccagccggaactgggcggctatcagattagcattccgcagaaaggcgtggtggataaacgtggcaaacgtaaaaaccgtccggcgcgtaaagcgagcctgagcctgcgtagcggccgtattaccctgaaacagggcaacattaccctgaacgcggtgctggccgaagaaattaatccgccgaaaggcgaaaccccgctgaaatggctgctgctgaccagcgagccggtggaaagtctggcccaagcgctgcgtgtgattgatatttatacccatcgttggcgcattgaagaatttcacaaagcgtggaaaacgggtgcgggtgcggaacgtcagcgtatggaagaaccggataacctggaacgtatggtgagcattctgagctttgtggcggtgcgtctgctgcaactgcgtgaatcttttactccgccgcaagcactgcgtgcgcagggcctgctgaaagaagcggaacacgttgaaagccagagcgcggaaaccgtgctgaccccggatgaatgccaactgctgggctatctggataaaggcaaacgcaaacgcaaagaaaaagcgggcagcctgcaatgggcgtatatggcgattgcgcgtctgggcggctttatggatagcaaacgtaccggcattgcgagctggggtgcgctgtgggaaggttgggaagcgctgcaaagcaaactggatggctttctggccgcgaaagacctgatggcgcagggcattaaaatctgcatcacgggagatgcactagttgccctacccgagggcgagtcggtacgcatcgccgacatcgtgccgggtgcgcggcccaacagtgacaacgccatcgacctgaaagtccttgaccggcatggcaatcccgtgctcgccgaccggctgttccactccggcgagcatccggtgtacacggtgcgtacggtcgaaggtctgcgtgtgacgggcaccgcgaaccacccgttgttgtgtttggtcgacgtcgccggggtgccgaccctgctgtggaagctgatcgacgaaatcaagccgggcgattacgcggtgattcaacgcagcgcattcagcgtcgactgtgcaggttttgcccgcgggaaacccgaatttgcgcccacaacctacacagtcggcgtccctggactggtgcgtttcttggaagcacaccaccgagacccggacgcccaagctatcgccgacgagctgaccgacgggcggttctactacgcgaaagtcgccagtgtcaccgacgccggcgtgcagccggtgtatagccttcgtgtcgacacggcagaccacgcgtttatcacgaacgggttcgtcagccacgctactggcctcaccggtctgaactcaggcctcacgacaaatcctggtgtatccgcttggcaggtcaacacagcttatactgcgggacaattggtcacatataacggcaagacgtataaatgtttgcagccccacacctccttggcaggatgggaaccatccaacgttcctgccttgtggcagcttcaatgactgcaggaaggggatccggctgctaacaaagcccgaaaggaagctgagttggctgctgccaccgctgagcaataactagcataaccccttggggcctctaaacgggtcttgaggggttttttgctgaaaggaggaactatatccggataactacgtcaggtggcacttttcggggaaatgtgcgcggaacccctatttgtttatttttctaaatacattcaaatatgtatccgctcatgagacaataaccctgataaatgcttcaataatattgaaaaaggaagagtatgagtattcaacatttccgtgtcgcccttattcccttttttgcggcattttgccttcctgtttttgctcacccagaaacgctggtgaaagtaaaagatgctgaagatcagttgggtgcacgagtgggttacatcgaactggatctcaacagcggtaagatccttgagagttttcgccccgaagaacgtttcccaatgatgagcacttttaaagttctgctatgtggcgcggtattatcccgtgttgacgccgggcaagagcaactcggtcgccgcatacactattctcagaatgacttggttgagtactcaccagtcacagaaaagcatcttacggatggcatgacagtaagagaattatgcagtgctgccataaccatgagtgataacactgcggccaacttacttctgacaacgatcggaggaccgaaggagctaaccgcttttttgcacaacatgggggatcatgtaactcgccttgatcgttgggaaccggagctgaatgaagccataccaaacgacgagcgtgacaccacgatgcctgtagcaatggcaacaacgttgcgcaaactattaactggcgaactacttactctagcttcccggcaacaattaatagactggatggaggcggataaagttgcaggaccacttctgcgctcggcccttccggctggctggtttattgctgataaatctggagccggtgagcgtgggtctcgcggtatcattgcagcactggggccagatggtaagccctcccgtatcgtagttatctacacgacggggagtcaggcaactatggatgaacgaaatagacagatcgctgagataggtgcctcactgattaagcattggtaactgtcagaccaagtttactcatatatactttagattgatttaccccggttgataatcagaaaagccccaaaaacaggaagattgtataagcaaatatttaaattgtaaacgttaatattttgttaaaattcgcgttaaatttttgttaaatcagctcattttttaaccaataggccgaaatcggcaaaatcccttataaatcaaaagaatagcccgagatagggttgagtgttgttccagtttggaacaagagtccactattaaagaacgtggactccaacgtcaaagggcgaaaaaccgtctatcagggcgatggcccactacgtgaaccatcacccaaatcaagttttttggggtcgaggtgccgtaaagcactaaatcggaaccctaaagggagcccccgatttagagcttgacggggaaagccggcgaacgtggcgagaaaggaagggaagaaagcgaaaggagcgggcgctagggcgctggcaagtgtagcggtcacgctgcgcgtaaccaccacacccgccgcgcttaatgcgccgctacagggcgcgtaaaaggatctaggtgaagatcctttttgataatctcatgaccaaaatcccttaacgtgagttttcgttccactgagcgtcagaccccgtagaaaagatcaaaggatcttcttgagatcctttttttctgcgcgtaatctgctgcttgcaaacaaaaaaaccaccgctaccagcggtggtttgtttgccggatcaagagctaccaactctttttccgaaggtaactggcttcagcagagcgcagataccaaatactgtccttctagtgtagccgtagttaggccaccacttcaagaactctgtagcaccgcctacatacctcgctctgctaatcctgttaccagtggctgctgccagtggcgataagtcgtgtcttaccgggttggactcaagacgatagttaccggataaggcgcagcggtcgggctgaacggggggttcgtgcacacagcccagcttggagcgaacgacctacaccgaactgagatacctacagcgtgagctatgagaaagcgccacgcttcccgaagggagaaaggcggacaggtatccggtaagcggcagggtcggaacaggagagcgcacgagggagcttccagggggaaacgcctggtatctttatagtcctgtcgggtttcgccacctctgacttgagcgtcgatttttgtgatgctcgtcaggggggcggagcctatggaaaaacgccagcaacgcggcctttttacggttcctggccttttgctggccttttgctcacatgttctttcctgcgttatcccctgattctgtggataaccgtattaccgcctttgagtgagctgataccgctcgccgcagccgaacgaccgagcgcagcgagtcagtgagcgaggaagctatggtgcactctcagtacaatctgctctgatgccgcatagttaagccagt

SEQ ID NO: 3 - DNA, 11245 bp, Artificial Sequence
  pET-Tn5-xTen-dCas9
caaggagatggcgcccaacagtcccccggccacggggcctgccaccatacccacgccgaaacaagcgctcatgagcccgaagtggcgagcccgatcttccccatcggtgatgtcggcgatataggcgccagcaaccgcacctgtggcgccggtgatgccggccacgatgcgtccggcgtagaggatcgagatctcgatcccgcgaaattaatacgactcactataggggaattgtgagcggataacaattcccctctagaaataattttgtttaactttaagaaggagatataccatgattaccagtgcactgcatcgtgcggcggattgggcgaaaagcgtgttttctagtgctgcgctgggtgatccgcgtcgtaccgcgcgtctggtgaatgttgcggcgcaactggccaaatatagcggcaaaagcattaccattagcagcgaaggcagcaaagccatgcaggaaggcgcgtatcgttttattcgtaatccgaacgtgagcgcggaagcgattcgtaaagcgggtgccatgcagaccgtgaaactggcccaggaatttccggaactgctggcaattgaagataccacctctctgagctatcgtcatcaggtggcggaagaactgggcaaactgggtagcattcaggataaaagccgtggttggtgggtgcatagcgtgctgctgctggaagcgaccacctttcgtaccgtgggcctgctgcatcaagaatggtggatgcgtccggatgatccggcggatgcggatgaaaaagaaagcggcaaatggctggccgctgctgcaacttcgcgtctgagaatgggcagcatgatgagcaacgtgattgcggtgtgcgatcgtgaagcggatattcatgcgtatctgcaagataaactggcccataacgaacgttttgtggtgcgtagcaaacatccgcgtaaagatgtggaaagcggcctgtatctgtatgatcacctgaaaaaccagccggaactgggcggctatcagattagcattccgcagaaaggcgtggtggataaacgtggcaaacgtaaaaaccgtccggcgcgtaaagcgagcctgagcctgcgtagcggccgtattaccctgaaacagggcaacattaccctgaacgcggtgctggccgaagaaattaatccgccgaaaggcgaaaccccgctgaaatggctgctgctgaccagcgagccggtggaaagtctggcccaagcgctgcgtgtgattgatatttatacccatcgttggcgcattgaagaatttcacaaagcgtggaaaacgggtgcgggtgcggaacgtcagcgtatggaagaaccggataacctggaacgtatggtgagcattctgagctttgtggcggtgcgtctgctgcaactgcgtgaatcttttactccgccgcaagcactgcgtgcgcagggcctgctgaaagaagcggaacacgttgaaagccagagcgcggaaaccgtgctgaccccggatgaatgccaactgctgggctatctggataaaggcaaacgcaaacgcaaagaaaaagcgggcagcctgcaatgggcgtatatggcgattgcgcgtctgggcggctttatggatagcaaacgtaccggcattgcgagctggggtgcgctgtgggaaggttgggaagcgctgcaaagcaaactggatggctttctggccgcgaaagacctgatggcgcagggcattaaaatcagcggttccgaaactcccggtacatcagaaagcgcgacccccgaaagcatggataaaaagtattctattggtttagctatcggcacaaatagcgtcggatgggcggtgatcactgatgaatataaggttccgtctaaaaagttcaaggttctgggaaatacagaccgccacagtatcaaaaaaaatcttataggggctcttttatttgacagtggagagacagcggaagcgactcgtctcaaacggacagctcgtagaaggtatacacgtcggaagaatcgtatttgttatctacaggagattttttcaaatgagatggcgaaagtagatgatagtttctttcatcgacttgaagagtcttttttggtggaagaagacaagaagcatgaacgtcatcctatttttggaaatatagtagatgaagttgcttatcatgagaaatatccaactatctatcatctgcgaaaaaaattggtagattctactgataaagcggatttgcgcttaatctatttggccttagcgcatatgattaagtttcgtggtcattttttgattgagggagatttaaatcctgataatagtgatgtggacaaactatttatccagttggtacaaacctacaatcaattatttgaagaaaaccctattaacgcaagtggagtagatgctaaagcgattctttctgcacgattgagtaaatcaagacgattagaaaatctcattgctcagctccccggtgagaagaaaaatggcttatttgggaatctcattgctttgtcattgggtttgacccctaattttaaatcaaattttgatttggcagaagatgctaaattacagctttcaaaagatacttacgatgatgatttagataatttattggcgcaaattggagatcaatatgctgatttgtttttggcagctaagaatttatcagatgctattttactttcagatatcctaagagtaaatactgaaataactaaggctcccctatcagcatcaatgattaaacgctacgatgaacatcatcaagacttgactcttttaaaagctttagttcgacaacaacttccagaaaagtataaagaaatcttttttgatcaatcaaaaaacggatatgcaggttatattgatgggggagctagccaagaagaattttataaatttatcaaaccaattttagaaaaaatggatggtactgaggaattattggtgaaactaaatcgtgaagatttgctgcgcaagcaacggacctttgacaacggctctattccccatcaaattcacttgggtgagctgcatgctattttgagaagacaagaagacttttatccatttttaaaagacaatcgtgagaagattgaaaaaatcttgacttttcgaattccttattatgttggtccattggcgcgtggcaatagtcgttttgcatggatgactcggaagtctgaagaaacaattaccccatggaattttgaagaagttgtcgataaaggtgcttcagctcaatcatttattgaacgcatgacaaactttgataaaaatcttccaaatgaaaaagtactaccaaaacatagtttgctttatgagtattttacggtttataacgaattgacaaaggtcaaatatgttactgaaggaatgcgaaaaccagcatttctttcaggtgaacagaagaaagccattgttgatttactcttcaaaacaaatcgaaaagtaaccgttaagcaattaaaagaagattatttcaaaaaaatagaatgttttgatagtgttgaaatttcaggagttgaagatagatttaatgcttcattaggtacctaccatgatttgctaaaaattattaaagataaagattttttggataatgaagaaaatgaagatatcttagaggatattgttttaacattgaccttatttgaagatagggagatgattgaggaaagacttaaaacatatgctcacctctttgatgataaggtgatgaaacagcttaaacgtcgccgttatactggttggggacgtttgtctcgaaaattgattaatggtattagggataagcaatctggcaaaacaatattagattttttgaaatcagatggttttgccaatcgcaattttatgcagctgatccatgatgatagtttgacatttaaagaagacattcaaaaagcacaagtgtctggacaaggcgatagtttacatgaacatattgcaaatttagctggtagccctgctattaaaaaaggtattttacagactgtaaaagttgttgatgaattggtcaaagtaatggggcggcataagccagaaaatatcgttattgaaatggcacgtgaaaatcagacaactcaaaagggccagaaaaattcgcgagagcgtatgaaacgaatcgaagaaggtatcaaagaattaggaagtcagattcttaaagagcatcctgttgaaaatactcaattgcaaaatgaaaagctctatctctattatctccaaaatggaagagacatgtatgtggaccaagaattagatattaatcgtttaagtgattatgatgtcgatgccattgttccacaaagtttccttaaagacgattcaatagacaataaggtcttaacgcgttctgataaaaatcgtggtaaatcggataacgttccaagtgaagaagtagtcaaaaagatgaaaaactattggagacaacttctaaacgccaagttaatcactcaacgtaagtttgataatttaacgaaagctgaacgtggaggtttgagtgaacttgataaagctggttttatcaaacgccaattggttgaaactcgccaaatcactaagcatgtggcacaaattttggatagtcgcatgaatactaaatacgatgaaaatgataaacttattcgagaggttaaagtgattaccttaaaatctaaattagtttctgacttccgaaaagatttccaattctataaagtacgtgagattaacaattaccatcatgcccatgatgcgtatctaaatgccgtcgttggaactgctttgattaagaaatatccaaaacttgaatcggagtttgtctatggtgattataaagtttatgatgttcgtaaaatgattgctaagtctgagcaagaaataggcaaagcaaccgcaaaatatttcttttactctaatatcatgaacttcttcaaaacagaaattacacttgcaaatggagagattcgcaaacgccctctaatcgaaactaatggggaaactggagaaattgtctgggataaagggcgagattttgccacagtgcgcaaagtattgtccatgccccaagtcaatattgtcaagaaaacagaagtacagacaggcggattctccaaggagtcaattttaccaaaaagaaattcggacaagcttattgctcgtaaaaaagactgggatccaaaaaaatatggtggttttgatagtccaacggtagcttattcagtcctagtggttgctaaggtggaaaaagggaaatcgaagaagttaaaatccgttaaagagttactagggatcacaattatggaaagaagttcctttgaaaaaaatccgattgactttttagaagctaaaggatataaggaagttaaaaaagacttaatcattaaactacctaaatatagtctttttgagttagaaaacggtcgtaaacggatgctggctagtgccggagaattacaaaaaggaaatgagctggctctgccaagcaaatatgtgaattttttatatttagctagtcattatgaaaagttgaagggtagtccagaagataacgaacaaaaacaattgtttgtggagcagcataagcattatttagatgagattattgagcaaatcagtgaattttctaagcgtgttattttagcagatgccaatttagataaagttcttagtgcatataacaaacatagagacaaaccaatacgtgaacaagcagaaaatattattcatttatttacgttgacgaatcttggagctcccgctgcttttaaatattttgatacaacaattgatcgtaaacgatatacgtctacaaaagaagttttagatgccactcttatccatcaatccatcactggtctttatgaaacacgcattgatttgagtcagctaggaggtgaccaccaccaccaccaccactgagatccggctgctaacaaagcccgaaaggaagctgagttggctgctgccaccgctgagcaataactagcataaccccttggggcctctaaacgggtcttgaggggttttttgctgaaaggaggaactatatccggatatcccgcaagaggcccggcagtaccggcataaccaagcctatgcctacagcatccagggtgacggtgccgaggatgacgatgagcgcattgttagatttcatacacggtgcctgactgcgttagcaatttaactgtgataaactaccgcattaaagctagcttatcgatgataagctgtcaaacatgagaattaattcttgaagacgaaagggcctcgtgatacgcctatttttataggttaatgtcatgataataatggtttcttagacgtcaggtggcacttttcggggaaatgtgcgcggaacccctatttgtttatttttctaaatacattcaaatatgtatccgctcatgagacaataaccctgataaatgcttcaataatattgaaaaaggaagagtatgagtattcaacatttccgtgtcgcccttattcccttttttgcggcattttgccttcctgtttttgctcacccagaaacgctggtgaaagtaaaagatgctgaagatcagttgggtgcacgagtgggttacatcgaactggatctcaacagcggtaagatccttgagagttttcgccccgaagaacgttttccaatgatgagcacttttaaagttctgctatgtggcgcggtattatcccgtgttgacgccgggcaagagcaactcggtcgccgcatacactattctcagaatgacttggttgagtactcaccagtcacagaaaagcatcttacggatggcatgacagtaagagaattatgcagtgctgccataaccatgagtgataacactgcggccaacttacttctgacaacgatcggaggaccgaaggagctaaccgcttttttgcacaacatgggggatcatgtaactcgccttgatcgttgggaaccggagctgaatgaagccataccaaacgacgagcgtgacaccacgatgcctgcagcaatggcaacaacgttgcgcaaactattaactggcgaactacttactctagcttcccggcaacaattaatagactggatggaggcggataaagttgcaggaccacttctgcgctcggcccttccggctggctggtttattgctgataaatctggagccggtgagcgtgggtctcgcggtatcattgcagcactggggccagatggtaagccctcccgtatcgtagttatctacacgacggggagtcaggcaactatggatgaacgaaatagacagatcgctgagataggtgcctcactgattaagcattggtaactgtcagaccaagtttactcatatatactttagattgatttaaaacttcatttttaatttaaaaggatctaggtgaagatcctttttgataatctcatgaccaaaatcccttaacgtgagttttcgttccactgagcgtcagaccccgtagaaaagatcaaaggatcttcttgagatcctttttttctgcgcgtaatctgctgcttgcaaacaaaaaaaccaccgctaccagcggtggtttgtttgccggatcaagagctaccaactctttttccgaaggtaactggcttcagcagagcgcagataccaaatactgtccttctagtgtagccgtagttaggccaccacttcaagaactctgtagcaccgcctacatacctcgctctgctaatcctgttaccagtggctgctgccagtggcgataagtcgtgtcttaccgggttggactcaagacgatagttaccggataaggcgcagcggtcgggctgaacggggggttcgtgcacacagcccagcttggagcgaacgacctacaccgaactgagatacctacagcgtgagctatgagaaagcgccacgcttcccgaagggagaaaggcggacaggtatccggtaagcggcagggtcggaacaggagagcgcacgagggagcttccagggggaaacgcctggtatctttatagtcctgtcgggtttcgccacctctgacttgagcgtcgatttttgtgatgctcgtcaggggggcggagcctatggaaaaacgccagcaacgcggcctttttacggttcctggccttttgctggccttttgctcacatgttctttcctgcgttatcccctgattctgtggataaccgtattaccgcctttgagtgagctgataccgctcgccgcagccgaacgaccgagcgcagcgagtcagtgagcgaggaagcggaagagcgcctgatgcggtattttctccttacgcatctgtgcggtatttcacaccgcaatggtgcactctcagtacaatctgctctgatgccgcatagttaagccagtatacactccgctatcgctacgtgactgggtcatggctgcgccccgacacccaccaacacccgctgacgcgccctgacgggcttgtctgctcccggcatccgcttacagacaagctgtgaccgtctccgggagctgcatgtgtcagaggttttcaccgtcatcaccgaaacgcgcgaggcagctgcggtaaagctcatcagcgtggtcgtgaagcgattcacagatgtctgcctgttcatccgcgtccagctcgttgagtttctccagaagcgttaatgtctggcttctgataaagcgggccatgttaagggcggttttttcctgtttggtcactgatgcctccgtgtaagggggatttctgttcatgggggtaatgataccgatgaaacgagagaggatgctcacgatacgggttactgatgatgaacatgcccggttactggaacgttgtgagggtaaacaactggcggtatggatgcggcgggaccagagaaaaatcactcagggtcaatgccagcgcttcgttaatacagatgtaggtgttccacagggtagccagcagcatcctgcgatgcagatccggaacataatggtgcagggcgctgacttccgcgtttccagactttacgaaacacggaaaccgaagaccattcatgttgttgctcaggtcgcagacgttttgcagcagcagtcgcttcacgttcgctcgcgtatcggtgattcattctgctaaccagtaaggcaaccccgccagcctagccgggtcctcaacgacaggagcacgatcatgcgcacccgtggccaggacccaacgctgcccgagatgcgccgcgtgcggctgctggagatggcggacgcgatggatatgttctgccaagggttggtttgcgcattcacagttctccgcaagaattgattggctccaattcttggagtggtgaatccgttagcgaggtgccgccggcttccattcaggtcgaggtggcccggctccatgcaccgcgacgcaacgcggggaggcagacaaggtatagggcggcgcctacaatccatgccaacccgttccatgtgctcgccgaggcggcataaatcgccgtgacgatcagcggtccaatgatcgaagttaggctggtaagagccgcgagcgatccttgaagctgtccctgatggtcgtcatctacctgcctggacagcatggcctgcaacgcgggcatcccgatgccgccggaagcgagaagaatcataatggggaaggccatccagcctcgcgtcgcgaacgccagcaagacgtagcccagcgcgtcggccgccatgccggcgataatggcctgcttctcgccgaaacgtttggtggcgggaccagtgacgaaggcttgagcgagggcgtgcaagattccgaataccgcaagcgacaggccgatcatcgtcgcgctccagcgaaagcggtcctcgccgaaaatgacccagagcgctgccggcacctgtcctacgagttgcatgataaagaagacagtcataagtgcggcgacgatagtcatgccccgcgcccaccggaaggagctgactgggttgaaggctctcaagggcatcggtcgagatcccggtgcctaatgagtgagctaacttacattaattgcgttgcgctcactgcccgctttccagtcgggaaacctgtcgtgccagctgcattaatgaatcggccaacgcgcggggagaggcggtttgcgtattgggcgccagggtggtttttcttttcaccagtgagacgggcaacagctgattgcccttcaccgcctggccctgagagagttgcagcaagcggtccacgctggtttgccccagcaggcgaaaatcctgtttgatggtggttaacggcgggatataacatgagctgtcttcggtatcgtcgtatcccactaccgagatatccgcaccaacgcgcagcccggactcggtaatggcgcgcattgcgcccagcgccatctgatcgttggcaaccagcatcgcagtgggaacgatgccctcattcagcatttgcatggtttgttgaaaaccggacatggcactccagtcgccttcccgttccgctatcggctgaatttgattgcgagtgagatatttatgccagccagccagacgcagacgcgccgagacagaacttaatgggcccgctaacagcgcgatttgctggtgacccaatgcgaccagatgctccacgcccagtcgcgtaccgtcttcatgggagaaaataatactgttgatgggtgtctggtcagagacatcaagaaataacgccggaacattagtgcaggcagcttccacagcaatggcatcctggtcatccagcggatagttaatgatcagcccactgacgcgttgcgcgagaagattgtgcaccgccgctttacaggcttcgacgccgcttcgttctaccatcgacaccaccacgctggcacccagttgatcggcgcgagatttaatcgccgcgacaatttgcgacggcgcgtgcagggccagactggaggtggcaacgccaatcagcaacgactgtttgcccgccagttgttgtgccacgcggttgggaatgtaattcagctccgccatcgccgcttccactttttcccgcgttttcgcagaaacgtggctggcctggttcaccacgcgggaaacggtctgataagagacaccggcatactctgcgacatcgtataacgttactggtttcacattcaccaccctgaattgactctcttccgggcgctatcatgccataccgcgaaaggttttgcgccattcgatggtgtccgggatctcgacgctctcccttatgcgactcctgcattaggaagcagcccagtagtaggttgaggccgttgagcaccgccgccgcaaggaatggtgcatg

SEQ ID NO: 4 - DNA, 20 bp, Artificial Sequence
  CD.Cas9.CVSJ0588.AF
gaaattaatggtttaagctt

SEQ ID NO: 5 - DNA, 20 bp, Artificial Sequence
  CD.Cas9.CVSJ0588.AA
aggtgagcaagatttccatt

SEQ ID NO: 6 - DNA, 20 bp, Artificial Sequence
  CD.Cas9.CVSJ0588.AC
tcaaggacatattctcctgt

SEQ ID NO: 7 - DNA, 20 bp, Artificial Sequence
  CD.Cas9.CVSJ0588.AJ
aatgtgctccataaggaatt

SEQ ID NO: 8 - DNA, 20 bp, Artificial Sequence
  CD.Cas9.CVSJ0588.AG
aactttcttcttctgaggag

SEQ ID NO: 9 - DNA, 20 bp, Artificial Sequence
  CD.Cas9.CVSJ0588.AB
aagatcacacctatgggaaa

SEQ ID NO: 10 - DNA, 20 bp, Artificial Sequence
  CD.Cas9.RNXS0617.AA
gctattttgaccatttcaat

SEQ ID NO: 11 - DNA, 20 bp, Artificial Sequence
  CD.Cas9.RNXS0617.AB
cggaggacaaatccatacca

SEQ ID NO: 12 - DNA, 20 bp, Artificial Sequence
  CD.Cas9.RNXS0617.AC
cagtttatcgttattaccaa

SEQ ID NO: 13 - DNA, 20 bp, Artificial Sequence
  CD.Cas9.RNXS0617.AD
acttataccatgctgaccat

SEQ ID NO: 14 - DNA, 20 bp, Artificial Sequence
  CD.Cas9.RZZJ8230.AA
ggacaacaccctgaccatcc

SEQ ID NO: 15 - DNA, 20 bp, Artificial Sequence
  CD.Cas9.RZZJ8230.AC
gtctgacctcgactccatcc

SEQ ID NO: 16 - DNA, 20 bp, Artificial Sequence
  CD.Cas9.RZZJ8230.AD
gaacatcaaaggtctgactc

SEQ ID NO: 17 - DNA, 20 bp, Artificial Sequence
  EXT1-1
atatcacgtccataacgggg

SEQ ID NO: 18 - DNA, 20 bp, Artificial Sequence
  EXT1-4
cacttggcctgactacaccg

SEQ ID NO: 19 - DNA, 20 bp, Artificial Sequence
  BCL9-2
gggttggcatcggaaccacg

SEQ ID NO: 20 - DNA, 20 bp, Artificial Sequence
  BCL9-4
gatgccctctccaaatgccg

SEQ ID NO: 21 - DNA, 20 bp, Artificial Sequence
  HOXA13-1
gtagccatagggcagcgccg

SEQ ID NO: 22 - DNA, 20 bp, Artificial Sequence
  HOXA13-4
tttctctacgacaacggcgg

SEQ ID NO: 23 - DNA, 20 bp, Artificial Sequence
  HOXD11-1
gggcttcgaccagttctacg

SEQ ID NO: 24 - DNA, 20 bp, Artificial Sequence
  HOXD11-3
gggctacgctccctactacg

SEQ ID NO: 25 - DNA, 20 bp, Artificial Sequence
  OLIG2-1
actggtgagcgagatctacg

SEQ ID NO: 26 - DNA, 20 bp, Artificial Sequence
  OLIG2-2
gcacgccgcacatcaccccg

SEQ ID NO: 27 - DNA, 33 bp, Artificial Sequence
  Adaptor A
tcgtcggcagcgtcagatgtgtataagagacag

SEQ ID NO: 28 - DNA, 34 bp, Artificial Sequence
  Adaptor B
gtctcgtgggctcggagatgtgtataagagacag

SEQ ID NO: 29 - DNA, 19 bp, Artificial Sequence
  Mosaic end
agatgtgtataagagacag

SEQ ID NO: 30 - DNA, 15 bp, Artificial Sequence
  Illumina Sequence Primer Site-SP2
gtctcgtgggctcgg

SEQ ID NO: 31 - DNA, 14 bp, Artificial Sequence
  Illumina Sequence Primer Site-SP1
tcgtcggcagcgtc

SEQ ID NO: 32 - protein, 10 aa, Artificial Sequence
  (G)n
  Variant (2)..(10): May be present or absent
GGGGGGGGGG

SEQ ID NO: 33 - protein, 20 aa, Artificial Sequence
  (GS)n
  Variant (3)..(20): May be present or absent
GSGSGSGSGSGSGSGSGSGS

SEQ ID NO: 34 - protein, 50 aa, Artificial Sequence
  (GSGGS)n
  Variant (6)..(50): May be present or absent
GSGGSGSGGSGSGGSGSGGSGSGGSGSGGSGSGGSGSGGSGSGGSGSGGS

SEQ ID NO: 35 - protein, 50 aa, Artificial Sequence
  (G4S)n
  Variant (6)..(50): May be present or absent
GGGGSGGGGSGGGGSGGGGSGGGGSGGGGSGGGGSGGGGSGGGGSGGGGS

SEQ ID NO: 36 - protein, 40 aa, Artificial Sequence
  (GGGS)n
  Variant (5)..(40): May be present or absent
GGGSGGGSGGGSGGGSGGGSGGGSGGGSGGGSGGGSGGGS

SEQ ID NO: 37 - protein, 4 aa, Artificial Sequence
  glycine/serine spacer 1
GGSG

SEQ ID NO: 38 - protein, 5 aa, Artificial Sequence
  glycine/serine spacer 2
GGSGG

SEQ ID NO: 39 - protein, 5 aa, Artificial Sequence
  glycine/serine spacer 3
GSGSG

SEQ ID NO: 40 - protein, 5 aa, Artificial Sequence
  glycine/serine spacer 4
GSGGG

SEQ ID NO: 41 - protein, 5 aa, Artificial Sequence
  glycine/serine spacer 5
GGGSG

SEQ ID NO: 42 - protein, 5 aa, Artificial Sequence
  glycine/serine spacer 6
GSSSG

SEQ ID NO: 43 - protein, 12 aa, Artificial Sequence
  XTEN linker 1
SGSETPGTSESA

SEQ ID NO: 44 - protein, 16 aa, Artificial Sequence
  XTEN linker 2
SGSETPGTSESATPES

SEQ ID NO: 45 - protein, 21 aa, Artificial Sequence
  XTEN linker 3
SGSETPGTSESATPEGGSGGS